European Patent Specification EP 3 980 244 B1, published May 27, 2026. Title: FUNCTIONAL MATERIALS WITH EMBEDDED MEMORY USING SEQUENCE-CONTROLLED POLYMER-BASED STORAGE. Applicant: ETH Zurich. The sequence listing filed with the application follows.

SEQUENCE LISTING (15 sequences)

SEQ ID NO: 1 - DNA, 20 bp, Artificial Sequence
  forward primer F0
acacgacgctcttccgatct

SEQ ID NO: 2 - DNA, 21 bp, Artificial Sequence
  backward primer R0
agacgtgtgctcggccgatct

SEQ ID NO: 3 - DNA, 33 bp, Artificial Sequence
  forward primer F1
acactctttccctacacgacgctcttccgatct

SEQ ID NO: 4 - DNA, 34 bp, Artificial Sequence
  backward primer R1
gtgactgcagttcagacgtgtgctcggccgatct

SEQ ID NO: 5 - DNA, 38 bp, Artificial Sequence
  forward primer 2FU
aatgatacggcgaccaccgagatctacactctttccct

SEQ ID NO: 6 - DNA, 58 bp, Artificial Sequence
  sequence comprising the primer sequence of Fig. 4A
aatgatacggcgaccaccgagatctacactctttccctacacgacgctcttccgatct

SEQ ID NO: 7 - DNA, 47 bp, Artificial Sequence
  Sequence of Fig. 4B comprising primer 2FU
aatgatacggcgaccaccgagatctacactctttccctacacgacgc

SEQ ID NO: 8 - DNA, 43 bp, Artificial Sequence
  backward primer "index" of Fig. 4A
caagcagaagacggcatacgagatcgtgatgtgactggagttc

SEQ ID NO: 9 - DNA, 64 bp, Artificial Sequence
  backward sequence of Fig. 4A comprising primer index
caagcagaagacggcatacgagatcgtgatgtgactggagttcagacgtgtgctcggccgatct

SEQ ID NO: 10 - DNA, 51 bp, Artificial Sequence
  backward sequence index 1 of Fig. 4B
caagcagaagacggcatacgagatcactgtgtgactggagttcagacgtgt

SEQ ID NO: 11 - DNA, 51 bp, Artificial Sequence
  backward sequence index 2 of Fig. 4B
caagcagaagacggcatacgagatattggcgtgactggagttcagacgtgt

SEQ ID NO: 12 - DNA, 51 bp, Artificial Sequence
  backward sequence index 3 of Fig. 4B
caagcagaagacggcatacgagatgatctggtgactggagttcagacgtgt

SEQ ID NO: 13 - DNA, 51 bp, Artificial Sequence
  backward sequence index 4 of Fig. 4B
caagcagaagacggcatacgagattcaagtgtgactggagttcagacgtgt

SEQ ID NO: 14 - DNA, 51 bp, Artificial Sequence
  backward sequence index 5 of Fig. 4B
caagcagaagacggcatacgagatctgatcgtgactggagttcagacgtgt

SEQ ID NO: 15 - DNA, 51 bp, Artificial Sequence
  backward sequence index 6 of Fig. 4B
caagcagaagacggcatacgagataagctagtgactggagttcagacgtgt